European Patent Specification EP 3 619 237 B1, published January 17, 2024. Title: ANTIBODIES AGAINST CARCINOEMBRYONIC ANTIGEN FOR CANCER THERAPY AND DIAGNOSIS. Applicant: B CELL DESIGN. The sequence listing filed with the application follows.

SEQUENCE LISTING (18 sequences)

SEQ ID NO: 1 - protein, 6 aa, artificial sequence
  synthetic peptide
QTIGTR

SEQ ID NO: 2 - protein, 9 aa, artificial sequence
  synthetic peptide
QQLYSTPYT

SEQ ID NO: 3 - protein, 8 aa, artificial sequence
  synthetic peptide
GYTFTNYG

SEQ ID NO: 4 - protein, 8 aa, artificial sequence
  synthetic peptide
INTNTGEP

SEQ ID NO: 5 - protein, 10 aa, artificial sequence
  synthetic peptide
ARLWYLYFDV

SEQ ID NO: 6 - protein, 6 aa, artificial sequence
  synthetic peptide
QSFSNN

SEQ ID NO: 7 - protein, 9 aa, artificial sequence
  synthetic peptide
QQSNSWPLT

SEQ ID NO: 8 - protein, 8 aa, artificial sequence
  synthetic peptide
GYTFTNYG

SEQ ID NO: 9 - protein, 8 aa, artificial sequence
  synthetic peptide
INTNTGEP

SEQ ID NO: 10 - protein, 10 aa, artificial sequence
  synthetic peptide
ARLWYLYFDV

SEQ ID NO: 11 - protein, 107 aa, artificial sequence
  synthetic polypeptide
DIQMTQSPASQSASLGESVTITCLASQTIGTRLAWYQQKPGKSPQLLIYAATRLADGVPSRFSGSGSGTKFSFKISSLQAEDFVSYYCQQLYSTPYTFGGGTKLEIK

SEQ ID NO: 12 - protein, 117 aa, artificial sequence
  synthetic polypeptide
QIQLVQSGPELKKPGETVKISCKASGYTFTNYGMNWVNQAPGKGLKWMGWINTNTGEPTYAEEFKGRFAFSLETSASTAYLQINNLKNEDTATYFCARLWYLYFDVWGAGTTVTVSS

SEQ ID NO: 13 - protein, 107 aa, artificial sequence
  synthetic polypeptide
DIVLTQSPATLSVTPGDSVSLSCRASQSFSNNLHWYQQKSHESPRLLIKYASQSISGIPSKFTGSGSGTDFTLSINSVETEDFGMYFCQQSNSWPLTFGAGTKLELK

SEQ ID NO: 14 - protein, 117 aa, artificial sequence; identical to SEQ ID NO: 12
  synthetic polypeptide

SEQ ID NO: 15 - DNA, 321 bp, artificial sequence
  synthetic polynucleotide
gacattcagatgacccagtctcctgcctcccagtctgcatctctgggagaaagtgtcaccatcacatgcctggcaagtcagaccattggtacacggttagcatggtatcagcagaaaccagggaaatctcctcagctcctgatttatgcagcaaccaggttggcagatggggtcccatcaaggttcagtggtagtggatctggcacaaaattttctttcaagatcagcagcctacaggctgaagattttgtaagttattactgtcaacaactttacagtactccgtacacgttcggaggggggaccaagctggaaataaaa

SEQ ID NO: 16 - DNA, 351 bp, artificial sequence
  synthetic polynucleotide
cagatccagttggtgcagtctggacctgagctgaagaagcctggagagacagtcaagatctcctgcaaggcttctgggtataccttcacaaactatggaatgaactgggtaaaccaggctccaggaaagggtttaaagtggatgggctggataaacaccaacactggagagccaacatatgctgaagagttcaagggacggtttgccttctctttggaaacctctgccagcactgcctatttgcagatcaacaacctcaaaaatgaggacacggctacatatttctgtgcaagattgtggtacctgtacttcgatgtctggggcgcagggaccacggtcaccgtctcctca

SEQ ID NO: 17 - DNA, 322 bp, artificial sequence
  synthetic polynucleotide
gatattgtgctaactcagtctccagccaccctgtctgtgactccaggagatagcgtcagtctttcctgcagggccagccaaagttttagcaacaacctacactggtatcaacaaaaatcacatgagtctccaaggcttctcatcaagtatgcttcccagtccatctctgggatcccctccaagttcactggcagtggatcagggacagatttcactctcagtatcaacagtgtggagactgaagattttggaatgtatttctgtcaacagagtaacagctggcctctcacgttcggtgctgggaccaagctggagttgaaac

SEQ ID NO: 18 - DNA, 351 bp, artificial sequence; identical to SEQ ID NO: 16
  synthetic polynucleotide